European Patent Specification EP 3 334 754 B1, published December 18, 2024. Title: COMPOSITIONS AND METHODS FOR FABRICATING SYNTHETIC DRAGLINE SPIDER SILK. Applicant: SEEVIX MATERIAL SCIENCES LTD. The sequence listing filed with the application follows.

SEQUENCE LISTING (47 sequences)

SEQ ID NO: 1 - protein, 28 aa, artificial
  synthetic
  MISC_FEATURE (1)..(1): X is A or G
  MISC_FEATURE (2)..(2): X is S or G
  MISC_FEATURE (10)..(10): X is G or E
  MISC_FEATURE (11)..(11): X is G, S or N
  MISC_FEATURE (12)..(12): X is Q or Y
  MISC_FEATURE (15)..(15): X is G or S
  MISC_FEATURE (17)..(17): X is P or R
  MISC_FEATURE (20)..(20): X is Y or Q
  MISC_FEATURE (27)..(27): X is G or S
  MISC_FEATURE (28)..(28): X is S or G
XXGPGGYGPXXXGPXGXGGXGPGGPGXX

SEQ ID NO: 2 - protein, 27 aa, artificial
  synthetic
SGPGGYGPGSQGPSGPGGYGPGGPGSS

SEQ ID NO: 3 - protein, 35 aa, artificial
  synthetic
AAAAAAAASGPGGYGPGSQGPSGPGGYGPGGPGSS

SEQ ID NO: 4 - protein, 35 aa, artificial
  synthetic
AAAAAAAASGPGGYGPENQGPSGPGGYGPGGPGSS

SEQ ID NO: 5 - protein, 40 aa, artificial
  synthetic
MSYYHHHHHHDYDIPTTENLYFQGAMDPEFKGLRRRAQLV

SEQ ID NO: 6 - protein, 49 aa, artificial
  synthetic
MSYYHHHHHHDYDIPTTENLYFQGAMDPEFKGLRRRAQLVRPLSNLDNA

SEQ ID NO: 7 - protein, 54 aa, artificial
  synthetic
MSYYHHHHHHDYDIPTTENLYFQGAMDPEFKGLRRRAQLVDPPGCRNSARAGSS

SEQ ID NO: 8 - protein, 28 aa, artificial
  synthetic
  MISC_FEATURE (1)..(1): X is A or G
  MISC_FEATURE (2)..(2): X is S or G
  misc_feature (10)..(10): Xaa can be any naturally occurring amino acid
  MISC_FEATURE (11)..(11): X is S or G
  MISC_FEATURE (12)..(12): X is Q or Y
  MISC_FEATURE (15)..(15): X is S or G
  MISC_FEATURE (17)..(17): X is P or R
  MISC_FEATURE (20)..(20): X is Y or Q
  MISC_FEATURE (27)..(27): X is G or S
  MISC_FEATURE (28)..(28): X is G or S
XXGPGGYGPXXXGPXGXGGXGPGGPGXX

SEQ ID NO: 9 - protein, 114 aa, artificial
  synthetic
GPSGPGAYGPSPSASASVAASRLSSPAASSRVSSAVSSLVSSGPTNGAAVSGALNSLVSQISASNPGLSGCDALVQALLELVSALVAILSSASIGQVNVSSVSQSTQMISQALS

SEQ ID NO: 10 - protein, 555 aa, artificial
  synthetic
AAAAAAASGSGGYGPENQGPSGPVAYGPGGPVSSAAAAAAAGSGPGGYGPENQGPSGPGGYGPGGSGSSAAAAAAAASGPGGYGPGSQGPSGPGGSGGYGPGSQGPSGPGASSAAAAAAAASGPGGYGPGSQGPSGPGAYGPGGPGSSAAASGPGGYGPGSQGPSGPGGSGGYGPGSQGPSGPGGPGASAAAAAAAAASGPGGYGPGSQGPSGPGAYGPGGPGSSAAASGPGGYGPGSQGPSGPGAYGPGGPGSSAAAAAAAGSGPGGYGPGNQGPSGPGGYGPGGPGSSAAAAAAASGPGGYGPGSQGPSGPGVYGPGGPGSSAAAAAAAGSGPGGYGPGNQGPSGPGGYGPGGSGSSAAAAAAAASGPGGYGPGSQGPSGPGGSGGYGPGSQGPSGPGASSAAAAAAAASGPGGYGPGSQGPSGPGAYGPGGPGSSAAASGPGGYGPGSQGPSGPGAYGPGGPGSSAAAAAAASGPGGYGPGSQGPSGPGGSRGYGPGSQGPGGPGASAAAAAAAAASGPGGYGPGSQGPSGPGYQGPSGPGAYGPSPSASAS

SEQ ID NO: 11 - protein, 6 aa, artificial
  synthetic
HHHHHH

SEQ ID NO: 12 - protein, 9 aa, artificial
  synthetic
YPYDVPDYA

SEQ ID NO: 13 - protein, 11 aa, artificial
  synthetic
MASMTGGQQMG

SEQ ID NO: 14 - protein, 35 aa, artificial
  synthetic
SGPGGYGPGSQGPSGPGGYGPGGPGSSAAAAAAAA

SEQ ID NO: 15 - DNA, 105 bp, Artificial
  Synthetic
tctggtcctggaggttatggcccaggaagccaaggaccatctggtccaggaggatatggtccaggcggacctggctctagtgcagcagctgccgcagcagctgca

SEQ ID NO: 16 - DNA, 28 bp, Artificial
  Synthetic
atatgctgcaggccctagtggtcctgga

SEQ ID NO: 17 - DNA, 20 bp, Artificial
  Synthetic
tcgacaagcttggtaccgca

SEQ ID NO: 18 - protein, 266 aa, artificial
  synthetic
GSAMGYLWIQGQGGYGGLGQGGYGQGAGSSAAAAAAAAAAAAGGQGGQGQGGYGQGSGGSAAAAAAAAAAAAAAAGRGQGGYGQGSGGNAAAAAAAAAAAAAAAGQGGQGGYGRQSQGAGSAAAAAAAAAAAAAAGSGQGGYGGQGQGGYGQSSASASAAASAASTVANSVSRLSSPSAVSRVSSAVSSLVSNGQVNMAALPNIISNISSSVSASAPGCEVIVQALLEVITALVQIVSSSSVGYINPSAVNQITNVVANAMAQVMG

SEQ ID NO: 19 - protein, 257 aa, artificial
  synthetic
GSAMASGQGGQGGQGQGGYGQGAGISAAAAAAAAAAAGAAAGRGQGGYGQGAGGNAAAAAAAAAAAAAAGQGGQGGYGGQGLGGYGQGAGSSAAAAAAAAGRGQSVYASGGAGQGGYGGLGGQGAGRGGQGAGAAAAAAGGSGQGGYGGVGSGASAASAAASRLSSPEASSRVSSAVSNLVSSGPTNSAALSSTISNVVSQIGASNPGLSGCDVLVQALLEVVSALIHILGSSSIGQVNYGSAGQATQLVGQSVYQA

SEQ ID NO: 20 - protein, 276 aa, artificial
  synthetic
GSAMGQGSGGNAAAAAAAAAAAAASGQGGQGGQGQGGYGQGAGISAAAAAAAAAAAGAAAGRGQGGYGQGAGGNAAAAAAAAAAAAAAGQGGQGGYGGQGLGGYGQGAGSSAAAAAAAAGRGQSVYASGGAGQGGYGGLGGQGAGRGGQGAGAAAAAAGGSGQGGYGGVGSGASAASAAASRLSSPEASSRVSSAVSNLVSSGPTNSAALSSTISNVVSQIGASNPGLSGCDVLVQALLEVVSALIHILGSSSIGQVNYGSAGQATQLVGQSVYQA

SEQ ID NO: 21 - protein, 269 aa, artificial
  synthetic
GSAMGYLWIQGQGGYGGLGQGGYGQGAGSSAAAAACCAAAAAGGQGGQGQGGYGQGSGGSAAAAAAAAAAAAAAAGRGQGGYGQGSGGNAAAAAAAAAAAAAAAGQGGQGGYGRQSQGAGSAAAAAAAAAAAAAAGSGQGGYGGQGQGGYGQSSASASAAASAASTVANSVSRLSSPSAVSRVSSAVSSLVSNGQVNMAALPNIISNISSSVSASAPGASGCEVIVQALLEVITALVQIVSSSSVGYINPSAVNQITNVVANAMAQVMG

SEQ ID NO: 22 - protein, 269 aa, artificial
  synthetic
GSAMGYLWIQGQGGYGGLGQGGYGQGAGSSAAAAAAAAAAAAGGQGGQGQGGYGQGSGGSAAAAAAAAAAAAAAAGRGQGGYGQGSGGNAAAAAAAAAAAAAAAGQGGQGGYGRQSQGAGSAAAAAACCAAAAAAGSGQGGYGGQGQGGYGQSSASASAAASAASTVANSVSRLSSPSAVSRVSSAVSSLVSNGQVNMAALPNIISNISSSVSASAPGASGCEVIVQALLEVITALVQIVSSSSVGYINPSAVNQITNVVANAMAQVMG

SEQ ID NO: 23 - protein, 217 aa, artificial
  synthetic
GSAMGYLWIQGQGGYGGLGQGGYGQGAGSSAAAAAAAAAAAAGGQGGQGQGGYGQGSGAAAAAAAAAAAAAAAGRGQGGYGQGSGGNAAAAAAAAAAAAAAAGQGGQGGYGRQSQGAGSAAAAAAAAAAAAAAGSGQGGYGGQGQGGYGQSSASASAAASAASTVANSVSRLSSPSAVSRVSSAVSSLVSNGQVNMAALPNIISVNVVANAMAQVMG

SEQ ID NO: 24 - protein, 3129 aa, artificial
  synthetic
MTWSTRLALSFLFVLCTQSLYALAQANTPWSSKANADAFINSFISAASNTGSFSQDQMEDMSLIGNTLMAAMDNMGGRITPSKLQALDMAFASSVAEIAASEGGDLGVTTNAIADALTSAFYQTTGVVNSRFISEIRSLIGMFAQASANDVYASAGSSGGGGYGASSASAASASAAAPSGVAYQAPAQAQISFTLRGQQPVSYGQGGAGPGGAGAAAAAAAAAGGAGQGGQGGYGQGGYGQGGAGQGGSGAAAAAAAAAGGTGQGGAGQGGAGAAAAAAAAAGGAGQGGQGGYGQGGYGQGGTGQGGAGAAAAAAAAGGAGQGGQGGYGQGGYGQGGYGQGGSGAAAAAAAAAGGAGQGGQGGYGQGGYGQGGAGQGGAGAAAAAAAAAGGAGQGGYGRGGAGQGGAAAAAAAAAGAGQGGYGGQGAGQGGSGAAAAAAAAGGAGQGGQGGYGQGGYGQGGSGAAAAAAAAGGAGQGGQGGYGQGGYGQGGAGQGGAGAAAAAAAAGGAGQGGQGGYGQGGYGQGGAGQGGAGAAAAAAAAGGAGQGGQGGYGQGGYGQGGAGQGGAGAAAAAAAAGGAGQGGQGGYGQGGYGQGGAGQGGAAAAAAAAAGGAGQGGYGRGGAGQGGAAAAAGAGQGGYGGQGAGQGGAGAAAAAAAAGGAGQGGQGGYGRGGYGQGGAGQGGAGAAAAAAAAGGAGQGGQGGYGQGGYGQGGAGQGGAAAAAAAAGGAGQGGYGRGGAGQGGAAAAAAAAAGAGQGGYGGQGAGQGGAGAAAAAAAAGGAGQGGQGDYGRGGYGQGGAGQGGAGAAAAAAAAGGAGQGGQGGYGQGGYGQGGAGQGGAAAAASAAAAGGAGQGGYGRGGAGQGGAAAAAGAGQGGYGGQGAGQGGAGAAAAAAAAGGAGQGGQGGYGRGGYGQGGAGQGGAGAAAAATAAGGAGQGGQGGYGQGGYGQGGAGQGGAAAAAAAAAGGAGQGGYGRGGAGQGGAAAAAAAAAGAGQGGYGGQGAGQGGAGAAAAAAGGAGQGGQGGYGRGGYGQGGAGQGGAGAAAAAAAAGGAGQGGQGGYGQGGYGQGGAGQGGAAAAAAAAAGGAGQGGYGRGGAGQGGAAAAAGAGQGGYGGQGAGQGGAGAAAAASRGAGQGGQGGYGRGGYGQGGAGQGGAGAAAAAAAAGGAGQGGQGGYGQGGYGQGGAGQGGAAAAAAAAGGAGQGGYGRGGAGQGGAAAAAGAGQGGYGGQGAGQGGAGAAAAAAAAGGAGQGGQGGYGRGGYGQGGAGQGGAGAAAAAAAAGGAGQGGQGGYGQGGYGQGGAGQGGAAAAAAAAAGGAGQGGYGRGGAGQGGAAAAAAAAAGSGQGGYGGQGAGQGGAGAAAAAAAAGGAGQGGQGGYGRGGYGQGGAGQGGAGAAAAAAAAGGAGQGGQGGYGQGGYGQGGAGQGGAAAAAAAAAAGGAGQGGYGRGGAGQGGAAAAAGAGQGGYGGQGAGQGGAGAAAAAAAAGGAGQGGQGGYGRGGYGQGGAGQGGAGTAAAAAAAGGAGQGGQGGYGQGGYGQGGAGQGGAAAAAAAAAGGAGQGGYGRGGAGQGGAAAAAAAAAGAGQGGYGGQGAGQGGAGAAAAAAAAGGAGQGGQGGYGRGGYGQGGAGQGGAGAAAAAAAAGGASQGGQGGYGQGDYGQGGAGQGGAAAAAAAAGGAGQGGYGRGGAGQGGAAAAAGAGQGGYGGQGAGQGGAGAAAAAAAAGGAGRGGQGGYGRGGYGQGGAGQGGAGAAAAAAAAGGAGQGGQGGYGQGGYGQGGTGQGGAAAAAAAAAGGAGQGGYGRGGAGQGGAAAAAAAAAGAGQGGYGGQGAGQGGAGAAAAAAAAGGAGQGGQGGYGRGGYGQGGAGQGGAGAAAAAAAAGGAGQGGQGGYGQGGYGQGGYGQGGAGQGGAAAAAAAAGGAGQGGYGRGGAGQGGAAAAAGAGQGGYGGQGAGQGGAGAAAAAAAAGGAGQGGQGGYGRGGYGQGGAGQGGAGAAAAAAAAGGAGQGGQGGYGQGGYGQGGAGQGGAAAAAAAAAGGAGQGGYGRGGAGQGGAAAAAAAAAGSGQGGYGGQGAGQGGAGAAAAAAAAGGAGQGGQGGYGRGGYGQGGAGQGGAGAAAAAAAAGGAGQGGQGGYGQGGYGQGGYGQGGAGQGGAAAAAAAAAAGGAGQGGYGRGGAGQGGAAAAAGAGQGGYGGQGAGQGGAGAAAAAAAAGGAGQGGQGGYGRGGYGQGGAGQGGAGAAAAAAAAGGAGQGGQGGYGQGGNGQGGAGQGGAAAAAAAAGGAGQGGYGRGGAGQGGAAAAAAAAAGAGQGGYGGQGAGQGGAGAAAAAAAAGGAGQGGQGGYGRGGYGQGGAGQGGAGAAAAAAAAGGASQGGQGGYGQGDYGQGGAGQGGAAAAAAAAGGAGQGGYGRGGAGQGGAAAAAGAGQGGYGGQGAGQGGAGAAAAAAAAGGAGRGGQGGYGRGGYGQGGAGQGGAGAAAAAAAAGGAGQGGQGGYGQGGYGQGGAGQGGAAAAAAAAAGGAGQGGYGRGGAGQGGAAAAAGAGQGGYGGQGAGQGGAGAAAAAAAAGGAGRGGQGGYGRGGYGQGGAGQGGAGAAAAAAAAGGAGQGGQGGYGQGGYGQGGAGQGGAAAAAAAAVGGAGQGGYGRGGAGQGGAAAAAAAAAAGSGQGGYGGQGAGQGGAGAAAAAAAAGGAGQGGQGGYGGGGYGQGGAGQGGAGAAAAAAAAGGAGQGGQGGYGQGGYGQGGAGQGGAAAAAAAAAGGAGQGGYGRGGAGQGGAAAATGAGQGGYGGQGAGQGGAGAAAAAAAAGGAGQGGQGGYGRGGYGQGGAGQGGAGAAAAAAAAGGAGQGGQGGYGQGGYGQGGAGQGGAAAAAAAAGGAGQGGYGRGGAGQGGAAAAAAAAAGAGQGGYGGQGAGQGGAGAAAAAAAAGGAGQGGQGGYGRGGYGQGGAGQGGAGAAAAGGAGQGGQGGYGQGGYGQGGAGQGGAAAAAAAAAAGGAGQGGYGGYGQQGGAGAAAAAASGPGQIYYGPQSVAAPAAAAASALAAPATSARISSHASALLSNGPTNPASISNVISNAVSQISSSNPGASACDVLVQALLELVTALLTIIGSSNIGSVNYDSSGQYAQVVTQSVQNAFA

SEQ ID NO: 25 - protein, 751 aa, artificial
  synthetic
MRRMYSLSIQSDFPTTTMTWSTRLALSFFAVICTQSIYALGQGNTPWSTKANADNFMNGFLSACAQSGVFSADQVDDMTTIGKTLMIAMDKMGGKISSSKLQALDMAFASSVAEIATAEGGANINDITDAIRYALQNAFYQTTGAVNSKFINEISNLIYMFAQTNINDVNGGGGYGQGGAGQGGAAAAAAGGAGQGGYGRGGARQGGAAAAAGAGQGGYGDQGAGQGGAGAAAAAATASGGAGQGGYGRGGAGQGGAAAAAAAAAGAGQGGYGGQGAAQGGAGAAAAAAAAGGAGLGGLGGYGQGGSGAAAAAGGAGQGGEGGVGQGGYGQRGAGQGGVGAAAAAAAAAGGAGQGEYGRGGAGKGGAAAAAAAAAGAGQGGYGGQGGAGAAAAAAAAGGAGLGGKGGYGQGGAGAAAAAAAAGGAGQGGQGGYGRGGYGRGGAGQGGAGAAAAAAAAGGAGQVGQSGYGQEGYGQGGAGQGGAGAAAAAAAAAGGAGQGGYGRGGAGQGEAAAAAAAAAGAGQGGYGGQGAGQGRAGAAAAAAAAGGAGQGGQGGYGQGGYGQGGSGAAAAAAAAAGGAGQGGQGGYGQGGYGQGGAGQGGAAAVAAAAAAGGAGQGGYGPQGGAGATAASASGPVQIYYGPQSVVAPAAAAASALAAPATSARISSHASALLSNGPTNPASISNVISNAVSQISSSNPGASACDVLVQALLELVTALLTIIGSSNIGSVNYDSSGQYAQVVTQSVQNAFA

SEQ ID NO: 26 - protein, 748 aa, artificial
  synthetic
MRRMYSLSIQSDFPTTTMTWSTRLALSFFAVICTQSIYALGQGNTPWSTKANADNFMNGFLSACAQSGVFSADQVDDMTTIGKTLMIAMDKMGGKISSSKLQALDMAFASSVAEIATAEGGANINDITDAIRYALQNAFYQTTGAVNSKFINEISNLIYFAQTNINDVNGGGGYGQGGAGQGGAAAAAAGGAGQGGYGRGGARQGGAAAAAGAGQGGYQGAGQGGAGAAAAAATASGGAGQGGYGRGGAGQGGAAAAAAAAAGAGQGGYGGQGAAQGGAGAAAAAAAAGGAGLGGLGGYGQGGSGAAAAAGGAGQGGEGGVGQGGYGQRGAGQGGVGAAAAAAAAAGGAGQGEYGRGGAGKGGAAAAAAAAAGAGQGGYGGQGGAGAAAAAAAAGGAGLGGKGGYGQGGAGAAAAAAAAGGAGQGGQGGYGRGGYGRGGAGQGGAGAAAAAAAAGGAGQVGQSGYGQEGYGQGGAGQGGAGAAAAAAAAAGGAGQGGYGRGGAGQGEAAAAAAAAAGAGQGGYGGQGAGQGRAGAAAAAAAAGGAGQGGQGGYGQGGYGQGGSGAAAAAAAAAGGAGQGGQGGYGQGGYGQGGAGQGGAAAVAAAAAAGGAGQGGYGPQGGAGATAASASGPVQIYYGPQSVVAPAAAAASALAAPATSARISSHASALLSNGPTNPASISNVISNAVSQISSSNPGASACDVLVQALLELVTALLTIIGSSNIGSVNYDSSGQYAQVVTQSVQNAFA

SEQ ID NO: 27 - protein, 631 aa, artificial
  synthetic
SRDFPTTTMTWSTRLALSFLFVLCTQSLYALAQANTPWSSKANADAFINSFISAASNTGSFSQDQMEDMSLIGNTLMAAMDNMGGRITPSKLQALDMAFASSVAEIAASEGGDLGVTTNAIADALTSAFYQTTGVVNSRFISEIRSLIGMFAQASANDVYASAGSSGGGGYGASSASAASASAAAPSGVAYQAPAQAQISFTLRGQQPVSYGQGGAGPGGAGAAAAAAAAAGGAGQGGQGGYGQGGYGQGGAGQGGSGAAAAAGGTGQGGAGQGGAGAAAAAAAAAGGAGQGGQGGYGQGGYGQGGTGQGGAGAAARGGYGQGGAGQGGAGAAAAAAAAGGAGQGGQGGYGQGGYGQGGAGQGGAAAAAAAAGGAGQGGYGRGGAGQGGAAAAAAAAAGAGQGGYGGQGAGQGGAGAAAAAAAAGGAGQGGQGGYGRGGYGQGGAGQGGAGAAAAAAAAAGGAGQGGQGGYGQGGYGQGGAGQGGAAAAAAAAAAGGAGQGGYGGYGQQGGAGAAAAAASGPGQIYYGPQSVAAPAAAAASALAAPATSARISSHASALLSNGPTNPASISNVISNAVSQISSSNPGASACDVLVQALLELVTALLTIIGSSNIGSVNYDSSGQYAQVVTQ

SEQ ID NO: 28 - protein, 697 aa, artificial
  synthetic
MYSLSIQSDFPTTTMTWSTRLALSFFAVICTQSIYALGQGNTPWSTKANADNFMNGFLSACAQSGVFSADQVDDMTTIGKTLMIAMDKMGGKISSSKLQALDMAFASSVAEIATAEGGANINDITDAIRYALQNAFYQTTGAVNSKFINEISNLIYMFAQTNINDVNGGGGYGQGGAGQGGAAAAAAGGAGQGGYGRGGAGQGGAAAAAGAGQGGYGDQGAGQGGAGAAAAAATASGGAGQGGYGRGGAGQGGEAAAAAAAAGAGQGGYGGQEAAQGGAGAAAAAAAAGGAGLGGLGGYGQGGSGAAAAAGGAGQGGEGGVGQGGYGQRGAGQGGAGAAAAAAGGAGQGEYGRGGAGQGRAAAAAAAAAGAGQGSYGGQGAGGYGRGGAGQGGAGAAAAAAAAGGAGQVGQSGYGQEGYGQGGAGQGGAGAAAAAAAAAGGAGQGGYGRGGAGQGGAAAAAAAAAGAGQGGYGGQGAGQGGAGAAAAAAAAGWAGQGGQGGYGQGGYGQGGSGAAAAAAAAAGGAGQGGQGGYGQGGYDQGGAGQGGAAAVAAAAAAGGAGQGGYGPQGGAGAAAASASGPVQIYYGPQSVAAPAAAAASALAAPATSARISSHASALLSNGPTNPASISNVISNAVSQISSSNPGASACDVLVQALLELVTALLTIIGSSNIGSVNYDSSGQYAQVVTQSVQNAFA

SEQ ID NO: 29 - protein, 675 aa, artificial
  synthetic
MTWSTRLALSFLLVLCTQSIYALAQANTPWSSKANADAFINSFISAASNTGSFSQDQMEDMSLIGNTLMAAMDNMGGRITPSKLQALDMAFASSVAEIAASEGGDLGVTTNAIADALTSAFYQTTGVVNSRFISEIRSLIGMFAQASANDVYASAGSSGGGGYGASSASAASASAAAPSGVAYQAPAQAQISFSLRGQQPVGYGQGGASAASGAAAGQGGAGPGGAGAAAAGGAGQGGQGGYGQGGYGQGGAGQGGSGAAAAAAAAAGGTGQGGAGQGGAGAAAAAAAAAGGAGQGGQGGYGQGGYGQGGSGAAAAAAAAAGGAGQGGQGDYGQGGYGQGGAGQGGAGAAAAAAAAAGGAGQGGYGRGAAAAAAAAGGAGQGGQGGYGQGGYGQGGSGAAAAAAAAAGGAGQGGQGGYGQGGYGQGGSGAAAAAAAAAGGAGQGGQGGYGQGGYGQGGAGQGGAGAAAAAAAAAGGAGQGGYGRGGAGQGGAAAAAAAAAGAGQRGYGGQGAGQGGAGAAAAAAAAGGAGQGGQRGYGQGGYGQGGSGAAAAAAAASGPGQVYYGPQSFAAPAAAAASALSAPATSARISSHASALLSSGPTNPASISNVISNAVSQISSSNPGASACDVLVQALLELVTALLTIIGSSNIGSVNYDSSGQYAQVVTQSVQNVFG

SEQ ID NO: 30 - protein, 605 aa, artificial
  synthetic
MTWSTRLALSFLFVLCTQSLYALAQANTPWSSKANADAFINSFISAASNTGSFSQDQMEDMSLIGNTLMAAMDNMGGRITPSKLQALDMAFASSVAEIAASEGGDLGVTTNAIADALTSAFYQTTGVVNSRFISEIRSLIGMFAQASANDVYASAGSSGGGGYGASSASAASASAAAPSGVAYQAPAQAQISFTLRGQQPVSYGQGGAGPGGAGAAAAAAAAAGGAGQGGQGGYGQGGYGQGGAGQGGSGAAAAAGGTGQGGAGQGGAGAAAAAAAAAGGAGQGGQGGYGQGGYGQGGTGQGGAGAAAAAAAAGGAGQGGQGGYGQGGYGQGGSGAAAAAAAAAGGAGQGGQGGYGQGGYGQGGAGQGGAGAAGQGGYGQGGYGQGGAGQGGAAAAAAAAGGAGQGGYGRGGAGQGGAAAAAAAAAGAGQGGYGGQGAGQGGAGAAAAAAAAGGAGQGGQGGYGRGGYDQGGAGQGGAGAAAAAAAAAGGAGQGGQGGYGQGGYGQGGAGQGGAAAAAAAAAAGGAGQGGYGGYGQQGGAGAAAAAASGPGQIYYGPQSVAAPAAAAASALAAPATSARISSHASALLSNGPTNPASISNVISNA

SEQ ID NO: 31 - protein, 729 aa, artificial
  synthetic
MTWSTRLALSFLFVLCTQSLYALAQANTPWSSKANADAFINSFISAASNTGSFSQDQMEDMSLIGNTLMAAMDNMGGRITPSKLQALDMAFASSVAEIAASEGGDLGVTTNAIADALTSAFYQTTGVVNSRFISEIRSLIGMFAQASANDVYASAGSSGGGGYGASSASAASASAAAPSGVAYQAPAQAQISFTLRGQQPVSYGQGGAGPGGAGAAAAAAAAAGGAGQGGQGGYGQGGYGQGGAGQGGSGAAAAAGGTGQGGAGQGGAGAAAAAAAAAGGAGQGGQGGYGQGGYGQGGTGQGGAGAAAAAAAAGGAGQGGQGGYGQGGYGQGGSGAAAAAAAAAGGAGQGGQGGYGQGGYGQGGAGQGGAGAAAAAAAAAGGAGQGGYGRGGAGQGGAAAAAAAAAGAGQGGYGGQGAGGAGAAAAAAAAGGAGQGGQGGYGQGGYGQGGAGQGGAAAAAAAAGGAGQGGYGRGGAGQGGAAAAAAAAAGAGQGGYGGQGAGQGGAGAAAAAAAAGGAGQGGQGGYGRGGYDQGGAGQGGAGAAAAAAAAAGGAGQGGQGGYGQGGYGQGGAGQGGAAAAAAAAAAGGAGQGGYGGYGQQGGAGAAAAAASGPGQIYYGPQSVAAPAAAAASALAAPATSARISSHASALLSNGPTNPASISNVISNAVSQISSSNPGASACDVLVQALLELVTALLTIIGSSNIGSVNYDSSGQYAQVVTQSVQNAFA

SEQ ID NO: 32 - protein, 285 aa, artificial
  synthetic
MTWSTRLALSFLLVLCTQSIYALAQANTPWSSKANADAFIGSFISSAQNTGAFSTDQMDDMSLIGNTLMAAMDNMGGRITPSKLQALDMAFASSVAEIAAAEGGDLGVTTNAIADALTSAFYQTTGVVNSRFISEIRSLINMFAQASANDVYASAGSSGGGGYGAASSSASAAASSSASAAAPSGVSYQAPAQAQISFSLTRQQQPVNYGQSGASAASAAAAGGAGQGGYGQGGAGQGGAGAAAAAAAAGGAGQGGQGGYGQGGAGQGGAAAAAAAAGGAGQGGQ

SEQ ID NO: 33 - protein, 22 aa, Artificial
  Synthetic peptide
  MISC_FEATURE (1)..(1): X is A or G
  MISC_FEATURE (2)..(2): X is SG or GG
  MISC_FEATURE (6)..(6): X is GQ or absent
  MISC_FEATURE (11)..(11): X is G or absent
  MISC_FEATURE (13)..(13): X is G or S
  MISC_FEATURE (17)..(17): X is SP or GR or absent
XXSGPXGGYGXPXQGPXGGYGP

SEQ ID NO: 34 - protein, 6 aa, Artificial
  Synthetic peptide
PGGYGP

SEQ ID NO: 35 - protein, 36 aa, Artificial
  Synthetic peptide
SGPGGYGPGSQGPSGPGGYGPGGPGSSAGAGAGAAA

SEQ ID NO: 36 - protein, 36 aa, Artificial
  Synthetic peptide
SGPGGYGPGSQGPSGPGGYGPGGPGSSAGAGAGAGA

SEQ ID NO: 37 - protein, 29 aa, Artificial
  Synthetic peptide
SGSGPGGYGPGGQGPGGYGPGGQGPYGPG

SEQ ID NO: 38 - protein, 36 aa, Artificial
  Synthetic peptide
SGSGPGGYGPGGQGPGGYGPGGQGPYGPGAAAAAAA

SEQ ID NO: 39 - protein, 29 aa, Artificial
  Synthetic peptide
GGSGPGGYGPGGQGPGGYGPGGQGPYGPG

SEQ ID NO: 40 - protein, 36 aa, Artificial
  Synthetic pepide
GGSGPGGYGPGGQGPGGYGPGGQGPYGPGAAAAAAA

SEQ ID NO: 41 - protein, 27 aa, Artificial
  Synthetic pepide
SGPGQGGYGGPGGQGPGRGGYGPGAGS

SEQ ID NO: 42 - protein, 36 aa, Artificial
  Synthetic pepide
SGPGQGGYGGPGGQGPGRGGYGPGAGSAAAAAAAAA

SEQ ID NO: 43 - protein, 37 aa, Artificial
  Synthetic pepide
ARTIFICIALGGPGQGGYGGPGGQGPGRGGYGPGAGS

SEQ ID NO: 44 - protein, 27 aa, Artificial
  Synthetic peptide
GGPGQGGYGGPGGQGPGRGGYGPGAGS

SEQ ID NO: 45 - DNA, 108 bp, Artificial
  Synthetic
tccggacccggtggctacggacctggttctcagggccccagcggaccaggtggctacggacctggtggcccaggatcctcagctggtgccggcgctggtgccgctgca

SEQ ID NO: 46 - DNA, 108 bp, Artificial
  Synthetic
tccggttctggccccggaggttacggccctggtggccagggaccaggtggctacggaccgggtggccaaggaccctacggtcctggcgctgccgctgccgcggctgca

SEQ ID NO: 47 - DNA, 108 bp, artificial
  Synthetic
tccggtccaggccaaggaggttacggcggacctggtggccagggacccggtcgtggcggatacggtccgggcgctggatctgctgccgcggcagctgccgcggctgca